European Patent Application EP 4 393 953 A1, published July 3, 2024. Title: Bispecific molecules specifically binding to B7-H3 and TGFβ and uses thereof. Applicant: 세라노틱스. The sequence listing filed with the application follows.

SEQUENCE LISTING (348 sequences)

SEQ ID NO: 1 - protein, 5 aa, synthetic construct
SYAMS

SEQ ID NO: 2 - protein, 5 aa, synthetic construct
  REGION 1..5: note = HCDR1
AYYMI

SEQ ID NO: 3 - protein, 5 aa, synthetic construct
  REGION 1..5: note = HCDR1
TYYMT

SEQ ID NO: 4 - protein, 5 aa, synthetic construct
SYGMH

SEQ ID NO: 5 - protein, 5 aa, synthetic construct
TYAMS

SEQ ID NO: 6 - protein, 5 aa, synthetic construct
TYAIS

SEQ ID NO: 7 - protein, 5 aa, synthetic construct
NFWIG

SEQ ID NO: 8 - protein, 5 aa, synthetic construct
SYWIS

SEQ ID NO: 9 - protein, 5 aa, synthetic construct
SYAMN

SEQ ID NO: 10 - protein, 17 aa, synthetic construct
TITGSGGSTYYADSVKG

SEQ ID NO: 11 - protein, 17 aa, synthetic construct
ITNPSGGVTSYAQKFQG

SEQ ID NO: 12 - protein, 17 aa, synthetic construct
IINPRGGSTSYAEKFQG

SEQ ID NO: 13 - protein, 17 aa, synthetic construct
AISGSGTSIYYANSVKS

SEQ ID NO: 14 - protein, 17 aa, synthetic construct
AISGSGGSTLYADSVKG

SEQ ID NO: 15 - protein, 16 aa, synthetic construct
SIYYSGYTHYNPSLES

SEQ ID NO: 16 - protein, 17 aa, synthetic construct
WINPPGSITSYADSVKG

SEQ ID NO: 17 - protein, 16 aa, synthetic construct
EISPSGNTNYNPSLKS

SEQ ID NO: 18 - protein, 17 aa, synthetic construct
TISGSGGQTYYADSVKG

SEQ ID NO: 19 - protein, 10 aa, synthetic construct
ARYKSGAFDI

SEQ ID NO: 20 - protein, 10 aa, synthetic construct
ARVGGRGFDI

SEQ ID NO: 21 - protein, 9 aa, synthetic construct
ARWNLGMDV

SEQ ID NO: 22 - protein, 9 aa, synthetic construct
ARGAGWFDY

SEQ ID NO: 23 - protein, 12 aa, synthetic construct
ARGGSATWAFDL

SEQ ID NO: 24 - protein, 10 aa, synthetic construct
ARGYSGWMDV

SEQ ID NO: 25 - protein, 10 aa, synthetic construct
AREVGDVLDY

SEQ ID NO: 26 - protein, 10 aa, synthetic construct
AREVGDLLDY

SEQ ID NO: 27 - protein, 11 aa, synthetic construct
ARWRSIWAFDY

SEQ ID NO: 28 - protein, 11 aa, synthetic construct
RASQGIGNYLG

SEQ ID NO: 29 - protein, 11 aa, synthetic construct
HASQGISNYVA

SEQ ID NO: 30 - protein, 11 aa, synthetic construct
RVSQSISSYLN

SEQ ID NO: 31 - protein, 13 aa, synthetic construct
SGSTSNIGSNTVN

SEQ ID NO: 32 - protein, 13 aa, synthetic construct
SGSSSNIGSNYVY

SEQ ID NO: 33 - protein, 11 aa, synthetic construct
GGNNIGSKSVH

SEQ ID NO: 34 - protein, 14 aa, synthetic construct
TGTSSDIGRYNYVS

SEQ ID NO: 35 - protein, 11 aa, synthetic construct
SGSNIGNNYVS

SEQ ID NO: 36 - protein, 11 aa, synthetic construct
SDNNIGSKSVH

SEQ ID NO: 37 - protein, 7 aa, synthetic construct
TASSLQS

SEQ ID NO: 38 - protein, 7 aa, synthetic construct
DASNRAT

SEQ ID NO: 39 - protein, 7 aa, synthetic construct
DASHRAT

SEQ ID NO: 40 - protein, 7 aa, synthetic construct
GKNIRPN

SEQ ID NO: 41 - protein, 7 aa, synthetic construct
RNNQRPS

SEQ ID NO: 42 - protein, 7 aa, synthetic construct
DNNKRPS

SEQ ID NO: 43 - protein, 7 aa, synthetic construct
RNTQRPS

SEQ ID NO: 44 - protein, 7 aa, synthetic construct
QDSKRPS

SEQ ID NO: 45 - protein, 10 aa, synthetic construct
QQGYSTPSWT

SEQ ID NO: 46 - protein, 9 aa, synthetic construct
QQSYSTLLT

SEQ ID NO: 47 - protein, 9 aa, synthetic construct
QQYYAPSVT

SEQ ID NO: 48 - protein, 11 aa, synthetic construct
QSYDSSLSGWV

SEQ ID NO: 49 - protein, 11 aa, synthetic construct
GTWDSSLSGVV

SEQ ID NO: 50 - protein, 11 aa, synthetic construct
AAWDDSLNVPV

SEQ ID NO: 51 - protein, 11 aa, synthetic construct
GTWDSSLNAYV

SEQ ID NO: 52 - protein, 11 aa, synthetic construct
LVWDRSSDHFV

SEQ ID NO: 53 - protein, 11 aa, synthetic construct
GTWDDSLSGPV

SEQ ID NO: 54 - protein, 30 aa, synthetic construct
QVQLVQSGAEVKKPGSSVKVSCKASGGTFS

SEQ ID NO: 55 - protein, 30 aa, synthetic construct
QVQLVQSGAEVKKPGASVKVSCKASGYTFT

SEQ ID NO: 56 - protein, 30 aa, synthetic construct
EVQLLESGGGLVQPGGSLRLSCAASGFTFS

SEQ ID NO: 57 - protein, 30 aa, synthetic construct
EVQLLESGGGLVQPGSSLRLSCAASGFTFS

SEQ ID NO: 58 - protein, 30 aa, synthetic construct
EVQLVESGGGLVQPGGSLRLSCAASGFTFS

SEQ ID NO: 59 - protein, 30 aa, synthetic construct
QVQLQQWGAGLLKPSETLSLTCAVYGGSFS

SEQ ID NO: 60 - protein, 30 aa, synthetic construct
QVQLQESGPGLVKPSETLSLTCTVSGGSIS

SEQ ID NO: 61 - protein, 30 aa, synthetic construct
EVQLVQSGAEVKKPGESLKISCKGSGYSFT

SEQ ID NO: 62 - protein, 30 aa, synthetic construct
QVQLQQSGPGLVKPSQTLSLTCAISGDSVS

SEQ ID NO: 63 - protein, 14 aa, synthetic construct
WVRQAPGQGLEWMG

SEQ ID NO: 64 - protein, 14 aa, synthetic construct
WVRQAPGKGLEWVS

SEQ ID NO: 65 - protein, 14 aa, synthetic construct
WIRQPPGKGLEWIG

SEQ ID NO: 66 - protein, 14 aa, synthetic construct
WVRQMPGKGLEWMG

SEQ ID NO: 67 - protein, 16 aa, synthetic construct
WNWIRQSPSRGLEWLG

SEQ ID NO: 68 - protein, 30 aa, synthetic construct
RVTITADESTSTAYMELSSLRSEDTAVYYC

SEQ ID NO: 69 - protein, 30 aa, synthetic construct
RVTMTTDTSTSTAYMELRSLRSDDTAVYYC

SEQ ID NO: 70 - protein, 30 aa, synthetic construct
RFTISRDNSKNTLYLQMNSLRAEDTAVYYC

SEQ ID NO: 71 - protein, 30 aa, synthetic construct
RFTISRDNSKDTLYLQMNSLRAEDTAVYYC

SEQ ID NO: 72 - protein, 30 aa, synthetic construct
RFTISRDNAKNSLYLQMNSLRDEDTAVYYC

SEQ ID NO: 73 - protein, 30 aa, synthetic construct
RVTISVDTSKNQFSLKLSSVTAADTAVYYC

SEQ ID NO: 74 - protein, 30 aa, synthetic construct
QVTISADKSISTAYLQWSSLKASDTAMYYC

SEQ ID NO: 75 - protein, 30 aa, synthetic construct
RITINPDTSKNQFSLQLNSVTPEDTAVYYC

SEQ ID NO: 76 - protein, 23 aa, synthetic construct
DIQMTQSPSSLSASVGDRVTITC

SEQ ID NO: 77 - protein, 23 aa, synthetic construct
DIQMTQSPSFLSASVGDRVTITC

SEQ ID NO: 78 - protein, 23 aa, synthetic construct
DIVMTQSPLSLPVTPGEPASISC

SEQ ID NO: 79 - protein, 23 aa, synthetic construct
EIVMTQSPATLSVSPGERATLSC

SEQ ID NO: 80 - protein, 23 aa, synthetic construct
EIVLTQSPGTLSLSPGERATLSC

SEQ ID NO: 81 - protein, 23 aa, synthetic construct
DIVMTQSPDSLAVSLGERATINC

SEQ ID NO: 82 - protein, 15 aa, synthetic construct
WYQQKPGKAPKLLIY

SEQ ID NO: 83 - protein, 15 aa, synthetic construct
WYLQKPGQSPQLLIY

SEQ ID NO: 84 - protein, 15 aa, synthetic construct
WYQQKPGQAPRLLIY

SEQ ID NO: 85 - protein, 15 aa, synthetic construct
WYQQKPGQPPKLLIY

SEQ ID NO: 86 - protein, 32 aa, synthetic construct
GVPSRFSGSGSGTDFTFTISSLQPEDIATYYC

SEQ ID NO: 87 - protein, 32 aa, synthetic construct
GVPSRFSGSGSGTDFTLTISSLQPEDFATYYC

SEQ ID NO: 88 - protein, 32 aa, synthetic construct
GVPDRFSGSGSGTDFTLKISRVEAEDVGVYYC

SEQ ID NO: 89 - protein, 32 aa, synthetic construct
GIPARFSGSGSGTEFTLTISSLQSEDFAVYYC

SEQ ID NO: 90 - protein, 32 aa, synthetic construct
GIPDRFSGSGSGTDFTLTISRLEPEDFAVYYC

SEQ ID NO: 91 - protein, 32 aa, synthetic construct
GIPDRFSGSGSGTDFTLTISHLEPEDFAVYYC

SEQ ID NO: 92 - protein, 32 aa, synthetic construct
GVPDRFSGSGSGTDFTLTISSLQAEDVAVYYC

SEQ ID NO: 93 - protein, 22 aa, synthetic construct
QSVLTQPPSASGTPGQRVTISC

SEQ ID NO: 94 - protein, 22 aa, synthetic construct
QSVLTQPPSVSAAPGQKVTISC

SEQ ID NO: 95 - protein, 22 aa, synthetic construct
QSALTQPASVSGSPGQSITISC

SEQ ID NO: 96 - protein, 22 aa, synthetic construct
QSALTQPRSVSGSPGQSVTISC

SEQ ID NO: 97 - protein, 22 aa, synthetic construct
SYELTQPPSVSVSPGQTASITC

SEQ ID NO: 98 - protein, 15 aa, synthetic construct
WYQQLPGTAPKLLIY

SEQ ID NO: 99 - protein, 15 aa, synthetic construct
WYQQHPGKAPKLMIY

SEQ ID NO: 100 - protein, 15 aa, synthetic construct
WYQQKPGQSPVLVIY

SEQ ID NO: 101 - protein, 32 aa, synthetic construct
GVPDRFSGSKSGTSASLAISGLQSEDEADYYC

SEQ ID NO: 102 - protein, 32 aa, synthetic construct
GVPDRFSGSKSGTSASLAISGLHSEDEADYYC

SEQ ID NO: 103 - protein, 32 aa, synthetic construct
GVPDRFSGSKSGTSASLAISGLRSEDEADYYC

SEQ ID NO: 104 - protein, 32 aa, synthetic construct
GVPNRFSGSKSGTSASLAISGLRSEDEADYYC

SEQ ID NO: 105 - protein, 32 aa, synthetic construct
GIPDRFSGSKSGTSATLGITGLQTGDEADYYC

SEQ ID NO: 106 - protein, 32 aa, synthetic construct
GVSNRFSGSKSGNTASLTISGLQAEDEADYYC

SEQ ID NO: 107 - protein, 32 aa, synthetic construct
GVPDRFSGSKSGNTASLTISGLQAEDEADYYC

SEQ ID NO: 108 - protein, 32 aa, synthetic construct
GIPERFSGSNSGNTATLTISGTQAMDEADYYC

SEQ ID NO: 109 - protein, 117 aa, synthetic construct
QVQLVQSGAEVKKPGSSVKVSCKASGGTFSSYAMSWVRQAPGQGLEWMGTITGSGGSTYYADSVKGRVTITADESTSTAYMELSSLRSEDTAVYYCARYKSGAFDIWGQGTLVTVSS

SEQ ID NO: 110 - protein, 117 aa, synthetic construct
QVQLVQSGAEVKKPGSSVKVSCKASGGTFSAYYMIWVRQAPGQGLEWMGITNPSGGVTSYAQKFQGRVTITADESTSTAYMELSSLRSEDTAVYYCARVGGRGFDIWGQGTLVTVSS

SEQ ID NO: 111 - protein, 116 aa, synthetic construct
QVQLVQSGAEVKKPGSSVKVSCKASGGTFSTYYMTWVRQAPGQGLEWMGIINPRGGSTSYAEKFQGRVTITADESTSTAYMELSSLRSEDTAVYYCARWNLGMDVWGQGTLVTVSS

SEQ ID NO: 112 - protein, 116 aa, synthetic construct
QVQLVQSGAEVKKPGSSVKVSCKASGGTFSSYGMHWVRQAPGQGLEWMGAISGSGTSIYYANSVKSRVTITADESTSTAYMELSSLRSEDTAVYYCARGAGWFDYWGQGTLVTVSS

SEQ ID NO: 113 - protein, 119 aa, synthetic construct
QVQLVQSGAEVKKPGSSVKVSCKASGGTFSTYAMSWVRQAPGQGLEWMGAISGSGGSTLYADSVKGRVTITADESTSTAYMELSSLRSEDTAVYYCARGGSATWAFDLWGQGTLVTVSS

SEQ ID NO: 114 - protein, 116 aa, synthetic construct
QVQLVQSGAEVKKPGSSVKVSCKASGGTFSTYAISWVRQAPGQGLEWMGSIYYSGYTHYNPSLESRVTITADESTSTAYMELSSLRSEDTAVYYCARGYSGWMDVWGQGTLVTVSS

SEQ ID NO: 115 - protein, 117 aa, synthetic construct
QVQLVQSGAEVKKPGSSVKVSCKASGGTFSNFWIGWVRQAPGQGLEWMGWINPPGSITSYADSVKGRVTITADESTSTAYMELSSLRSEDTAVYYCAREVGDVLDYWGQGTLVTVSS

SEQ ID NO: 116 - protein, 116 aa, synthetic construct
QVQLVQSGAEVKKPGSSVKVSCKASGGTFSSYWISWVRQAPGQGLEWMGEISPSGNTNYNPSLKSRVTITADESTSTAYMELSSLRSEDTAVYYCAREVGDLLDYWGQGTLVTVSS

SEQ ID NO: 117 - protein, 118 aa, synthetic construct
QVQLVQSGAEVKKPGSSVKVSCKASGGTFSSYAMNWVRQAPGQGLEWMGTISGSGGQTYYADSVKGRVTITADESTSTAYMELSSLRSEDTAVYYCARWRSIWAFDYWGQGTLVTVSS

SEQ ID NO: 118 - protein, 117 aa, synthetic construct
QVQLVQSGAEVKKPGASVKVSCKASGYTFTSYAMSWVRQAPGQGLEWMGTITGSGGSTYYADSVKGRVTMTTDTSTSTAYMELRSLRSDDTAVYYCARYKSGAFDIWGQGTLVTVSS

SEQ ID NO: 119 - protein, 117 aa, synthetic construct
QVQLVQSGAEVKKPGASVKVSCKASGYTFTAYYMIWVRQAPGQGLEWMGITNPSGGVTSYAQKFQGRVTMTTDTSTSTAYMELRSLRSDDTAVYYCARVGGRGFDIWGQGTLVTVSS

SEQ ID NO: 120 - protein, 116 aa, synthetic construct
QVQLVQSGAEVKKPGASVKVSCKASGYTFTTYYMTWVRQAPGQGLEWMGIINPRGGSTSYAEKFQGRVTMTTDTSTSTAYMELRSLRSDDTAVYYCARWNLGMDVWGQGTLVTVSS

SEQ ID NO: 121 - protein, 116 aa, synthetic construct
QVQLVQSGAEVKKPGASVKVSCKASGYTFTSYGMHWVRQAPGQGLEWMGAISGSGTSIYYANSVKSRVTMTTDTSTSTAYMELRSLRSDDTAVYYCARGAGWFDYWGQGTLVTVSS

SEQ ID NO: 122 - protein, 119 aa, synthetic construct
QVQLVQSGAEVKKPGASVKVSCKASGYTFTTYAMSWVRQAPGQGLEWMGAISGSGGSTLYADSVKGRVTMTTDTSTSTAYMELRSLRSDDTAVYYCARGGSATWAFDLWGQGTLVTVSS

SEQ ID NO: 123 - protein, 116 aa, synthetic construct
QVQLVQSGAEVKKPGASVKVSCKASGYTFTTYAISWVRQAPGQGLEWMGSIYYSGYTHYNPSLESRVTMTTDTSTSTAYMELRSLRSDDTAVYYCARGYSGWMDVWGQGTLVTVSS

SEQ ID NO: 124 - protein, 117 aa, synthetic construct
QVQLVQSGAEVKKPGASVKVSCKASGYTFTNFWIGWVRQAPGQGLEWMGWINPPGSITSYADSVKGRVTMTTDTSTSTAYMELRSLRSDDTAVYYCAREVGDVLDYWGQGTLVTVSS

SEQ ID NO: 125 - protein, 116 aa, synthetic construct
QVQLVQSGAEVKKPGASVKVSCKASGYTFTSYWISWVRQAPGQGLEWMGEISPSGNTNYNPSLKSRVTMTTDTSTSTAYMELRSLRSDDTAVYYCAREVGDLLDYWGQGTLVTVSS

SEQ ID NO: 126 - protein, 118 aa, synthetic construct
QVQLVQSGAEVKKPGASVKVSCKASGYTFTSYAMNWVRQAPGQGLEWMGTISGSGGQTYYADSVKGRVTMTTDTSTSTAYMELRSLRSDDTAVYYCARWRSIWAFDYWGQGTLVTVSS

SEQ ID NO: 127 - protein, 117 aa, synthetic construct
EVQLLESGGGLVQPGGSLRLSCAASGFTFSSYAMSWVRQAPGKGLEWVSTITGSGGSTYYADSVKGRFTISRDNSKNTLYLQMNSLRAEDTAVYYCARYKSGAFDIWGQGTLVTVSS

SEQ ID NO: 128 - protein, 117 aa, synthetic construct
EVQLLESGGGLVQPGGSLRLSCAASGFTFSAYYMIWVRQAPGKGLEWVSITNPSGGVTSYAQKFQGRFTISRDNSKNTLYLQMNSLRAEDTAVYYCARVGGRGFDIWGQGTLVTVSS

SEQ ID NO: 129 - protein, 116 aa, synthetic construct
EVQLLESGGGLVQPGGSLRLSCAASGFTFSTYYMTWVRQAPGKGLEWVSIINPRGGSTSYAEKFQGRFTISRDNSKNTLYLQMNSLRAEDTAVYYCARWNLGMDVWGQGTLVTVSS

SEQ ID NO: 130 - protein, 116 aa, synthetic construct
EVQLLESGGGLVQPGGSLRLSCAASGFTFSSYGMHWVRQAPGKGLEWVSAISGSGTSIYYANSVKSRFTISRDNSKNTLYLQMNSLRAEDTAVYYCARGAGWFDYWGQGTLVTVSS

SEQ ID NO: 131 - protein, 119 aa, synthetic construct
EVQLLESGGGLVQPGGSLRLSCAASGFTFSTYAMSWVRQAPGKGLEWVSAISGSGGSTLYADSVKGRFTISRDNSKNTLYLQMNSLRAEDTAVYYCARGGSATWAFDLWGQGTLVTVSS

SEQ ID NO: 132 - protein, 116 aa, synthetic construct
EVQLLESGGGLVQPGGSLRLSCAASGFTFSTYAISWVRQAPGKGLEWVSSIYYSGYTHYNPSLESRFTISRDNSKNTLYLQMNSLRAEDTAVYYCARGYSGWMDVWGQGTLVTVSS

SEQ ID NO: 133 - protein, 117 aa, synthetic construct
EVQLLESGGGLVQPGGSLRLSCAASGFTFSNFWIGWVRQAPGKGLEWVSWINPPGSITSYADSVKGRFTISRDNSKNTLYLQMNSLRAEDTAVYYCAREVGDVLDYWGQGTLVTVSS

SEQ ID NO: 134 - protein, 116 aa, synthetic construct
EVQLLESGGGLVQPGGSLRLSCAASGFTFSSYWISWVRQAPGKGLEWVSEISPSGNTNYNPSLKSRFTISRDNSKNTLYLQMNSLRAEDTAVYYCAREVGDLLDYWGQGTLVTVSS

SEQ ID NO: 135 - protein, 118 aa, synthetic construct
EVQLLESGGGLVQPGGSLRLSCAASGFTFSSYAMNWVRQAPGKGLEWVSTISGSGGQTYYADSVKGRFTISRDNSKNTLYLQMNSLRAEDTAVYYCARWRSIWAFDYWGQGTLVTVSS

SEQ ID NO: 136 - protein, 117 aa, synthetic construct
EVQLLESGGGLVQPGGSLRLSCAASGFTFSSYAMSWVRQAPGKGLEWVSTITGSGGSTYYADSVKGRFTISRDNSKDTLYLQMNSLRAEDTAVYYCARYKSGAFDIWGQGTLVTVSS

SEQ ID NO: 137 - protein, 117 aa, synthetic construct
EVQLLESGGGLVQPGGSLRLSCAASGFTFSAYYMIWVRQAPGKGLEWVSITNPSGGVTSYAQKFQGRFTISRDNSKDTLYLQMNSLRAEDTAVYYCARVGGRGFDIWGQGTLVTVSS

SEQ ID NO: 138 - protein, 116 aa, synthetic construct
EVQLLESGGGLVQPGGSLRLSCAASGFTFSTYYMTWVRQAPGKGLEWVSIINPRGGSTSYAEKFQGRFTISRDNSKDTLYLQMNSLRAEDTAVYYCARWNLGMDVWGQGTLVTVSS

SEQ ID NO: 139 - protein, 116 aa, synthetic construct
EVQLLESGGGLVQPGGSLRLSCAASGFTFSSYGMHWVRQAPGKGLEWVSAISGSGTSIYYANSVKSRFTISRDNSKDTLYLQMNSLRAEDTAVYYCARGAGWFDYWGQGTLVTVSS

SEQ ID NO: 140 - protein, 119 aa, synthetic construct
EVQLLESGGGLVQPGGSLRLSCAASGFTFSTYAMSWVRQAPGKGLEWVSAISGSGGSTLYADSVKGRFTISRDNSKDTLYLQMNSLRAEDTAVYYCARGGSATWAFDLWGQGTLVTVSS

SEQ ID NO: 141 - protein, 116 aa, synthetic construct
EVQLLESGGGLVQPGGSLRLSCAASGFTFSTYAISWVRQAPGKGLEWVSSIYYSGYTHYNPSLESRFTISRDNSKDTLYLQMNSLRAEDTAVYYCARGYSGWMDVWGQGTLVTVSS

SEQ ID NO: 142 - protein, 117 aa, synthetic construct
EVQLLESGGGLVQPGGSLRLSCAASGFTFSNFWIGWVRQAPGKGLEWVSWINPPGSITSYADSVKGRFTISRDNSKDTLYLQMNSLRAEDTAVYYCAREVGDVLDYWGQGTLVTVSS

SEQ ID NO: 143 - protein, 116 aa, synthetic construct
EVQLLESGGGLVQPGGSLRLSCAASGFTFSSYWISWVRQAPGKGLEWVSEISPSGNTNYNPSLKSRFTISRDNSKDTLYLQMNSLRAEDTAVYYCAREVGDLLDYWGQGTLVTVSS

SEQ ID NO: 144 - protein, 118 aa, synthetic construct
EVQLLESGGGLVQPGGSLRLSCAASGFTFSSYAMNWVRQAPGKGLEWVSTISGSGGQTYYADSVKGRFTISRDNSKDTLYLQMNSLRAEDTAVYYCARWRSIWAFDYWGQGTLVTVSS

SEQ ID NO: 145 - protein, 117 aa, synthetic construct
EVQLLESGGGLVQPGSSLRLSCAASGFTFSSYAMSWVRQAPGKGLEWVSTITGSGGSTYYADSVKGRFTISRDNSKNTLYLQMNSLRAEDTAVYYCARYKSGAFDIWGQGTLVTVSS

SEQ ID NO: 146 - protein, 117 aa, synthetic construct
EVQLLESGGGLVQPGSSLRLSCAASGFTFSAYYMIWVRQAPGKGLEWVSITNPSGGVTSYAQKFQGRFTISRDNSKNTLYLQMNSLRAEDTAVYYCARVGGRGFDIWGQGTLVTVSS

SEQ ID NO: 147 - protein, 116 aa, synthetic construct
EVQLLESGGGLVQPGSSLRLSCAASGFTFSTYYMTWVRQAPGKGLEWVSIINPRGGSTSYAEKFQGRFTISRDNSKNTLYLQMNSLRAEDTAVYYCARWNLGMDVWGQGTLVTVSS

SEQ ID NO: 148 - protein, 116 aa, synthetic construct
EVQLLESGGGLVQPGSSLRLSCAASGFTFSSYGMHWVRQAPGKGLEWVSAISGSGTSIYYANSVKSRFTISRDNSKNTLYLQMNSLRAEDTAVYYCARGAGWFDYWGQGTLVTVSS

SEQ ID NO: 149 - protein, 119 aa, synthetic construct
EVQLLESGGGLVQPGSSLRLSCAASGFTFSTYAMSWVRQAPGKGLEWVSAISGSGGSTLYADSVKGRFTISRDNSKNTLYLQMNSLRAEDTAVYYCARGGSATWAFDLWGQGTLVTVSS

SEQ ID NO: 150 - protein, 116 aa, synthetic construct
EVQLLESGGGLVQPGSSLRLSCAASGFTFSTYAISWVRQAPGKGLEWVSSIYYSGYTHYNPSLESRFTISRDNSKNTLYLQMNSLRAEDTAVYYCARGYSGWMDVWGQGTLVTVSS

SEQ ID NO: 151 - protein, 117 aa, synthetic construct
EVQLLESGGGLVQPGSSLRLSCAASGFTFSNFWIGWVRQAPGKGLEWVSWINPPGSITSYADSVKGRFTISRDNSKNTLYLQMNSLRAEDTAVYYCAREVGDVLDYWGQGTLVTVSS

SEQ ID NO: 152 - protein, 116 aa, synthetic construct
EVQLLESGGGLVQPGSSLRLSCAASGFTFSSYWISWVRQAPGKGLEWVSEISPSGNTNYNPSLKSRFTISRDNSKNTLYLQMNSLRAEDTAVYYCAREVGDLLDYWGQGTLVTVSS

SEQ ID NO: 153 - protein, 118 aa, synthetic construct
EVQLLESGGGLVQPGSSLRLSCAASGFTFSSYAMNWVRQAPGKGLEWVSTISGSGGQTYYADSVKGRFTISRDNSKNTLYLQMNSLRAEDTAVYYCARWRSIWAFDYWGQGTLVTVSS

SEQ ID NO: 154 - protein, 117 aa, synthetic construct
EVQLVESGGGLVQPGGSLRLSCAASGFTFSSYAMSWVRQAPGKGLEWVSTITGSGGSTYYADSVKGRFTISRDNAKNSLYLQMNSLRDEDTAVYYCARYKSGAFDIWGQGTLVTVSS

SEQ ID NO: 155 - protein, 117 aa, synthetic construct
EVQLVESGGGLVQPGGSLRLSCAASGFTFSAYYMIWVRQAPGKGLEWVSITNPSGGVTSYAQKFQGRFTISRDNAKNSLYLQMNSLRDEDTAVYYCARVGGRGFDIWGQGTLVTVSS

SEQ ID NO: 156 - protein, 116 aa, synthetic construct
EVQLVESGGGLVQPGGSLRLSCAASGFTFSTYYMTWVRQAPGKGLEWVSIINPRGGSTSYAEKFQGRFTISRDNAKNSLYLQMNSLRDEDTAVYYCARWNLGMDVWGQGTLVTVSS

SEQ ID NO: 157 - protein, 116 aa, synthetic construct
EVQLVESGGGLVQPGGSLRLSCAASGFTFSSYGMHWVRQAPGKGLEWVSAISGSGTSIYYANSVKSRFTISRDNAKNSLYLQMNSLRDEDTAVYYCARGAGWFDYWGQGTLVTVSS

SEQ ID NO: 158 - protein, 119 aa, synthetic construct
EVQLVESGGGLVQPGGSLRLSCAASGFTFSTYAMSWVRQAPGKGLEWVSAISGSGGSTLYADSVKGRFTISRDNAKNSLYLQMNSLRDEDTAVYYCARGGSATWAFDLWGQGTLVTVSS

SEQ ID NO: 159 - protein, 116 aa, synthetic construct
EVQLVESGGGLVQPGGSLRLSCAASGFTFSTYAISWVRQAPGKGLEWVSSIYYSGYTHYNPSLESRFTISRDNAKNSLYLQMNSLRDEDTAVYYCARGYSGWMDVWGQGTLVTVSS

SEQ ID NO: 160 - protein, 117 aa, synthetic construct
EVQLVESGGGLVQPGGSLRLSCAASGFTFSNFWIGWVRQAPGKGLEWVSWINPPGSITSYADSVKGRFTISRDNAKNSLYLQMNSLRDEDTAVYYCAREVGDVLDYWGQGTLVTVSS

SEQ ID NO: 161 - protein, 116 aa, synthetic construct
EVQLVESGGGLVQPGGSLRLSCAASGFTFSSYWISWVRQAPGKGLEWVSEISPSGNTNYNPSLKSRFTISRDNAKNSLYLQMNSLRDEDTAVYYCAREVGDLLDYWGQGTLVTVSS

SEQ ID NO: 162 - protein, 118 aa, synthetic construct
EVQLVESGGGLVQPGGSLRLSCAASGFTFSSYAMNWVRQAPGKGLEWVSTISGSGGQTYYADSVKGRFTISRDNAKNSLYLQMNSLRDEDTAVYYCARWRSIWAFDYWGQGTLVTVSS

SEQ ID NO: 163 - protein, 117 aa, synthetic construct
QVQLQQWGAGLLKPSETLSLTCAVYGGSFSSYAMSWIRQPPGKGLEWIGTITGSGGSTYYADSVKGRVTISVDTSKNQFSLKLSSVTAADTAVYYCARYKSGAFDIWGQGTLVTVSS

SEQ ID NO: 164 - protein, 117 aa, synthetic construct
QVQLQQWGAGLLKPSETLSLTCAVYGGSFSAYYMIWIRQPPGKGLEWIGITNPSGGVTSYAQKFQGRVTISVDTSKNQFSLKLSSVTAADTAVYYCARVGGRGFDIWGQGTLVTVSS

SEQ ID NO: 165 - protein, 116 aa, synthetic construct
QVQLQQWGAGLLKPSETLSLTCAVYGGSFSTYYMTWIRQPPGKGLEWIGIINPRGGSTSYAEKFQGRVTISVDTSKNQFSLKLSSVTAADTAVYYCARWNLGMDVWGQGTLVTVSS

SEQ ID NO: 166 - protein, 116 aa, synthetic construct
QVQLQQWGAGLLKPSETLSLTCAVYGGSFSSYGMHWIRQPPGKGLEWIGAISGSGTSIYYANSVKSRVTISVDTSKNQFSLKLSSVTAADTAVYYCARGAGWFDYWGQGTLVTVSS

SEQ ID NO: 167 - protein, 119 aa, synthetic construct
QVQLQQWGAGLLKPSETLSLTCAVYGGSFSTYAMSWIRQPPGKGLEWIGAISGSGGSTLYADSVKGRVTISVDTSKNQFSLKLSSVTAADTAVYYCARGGSATWAFDLWGQGTLVTVSS

SEQ ID NO: 168 - protein, 116 aa, synthetic construct
QVQLQQWGAGLLKPSETLSLTCAVYGGSFSTYAISWIRQPPGKGLEWIGSIYYSGYTHYNPSLESRVTISVDTSKNQFSLKLSSVTAADTAVYYCARGYSGWMDVWGQGTLVTVSS

SEQ ID NO: 169 - protein, 117 aa, synthetic construct
QVQLQQWGAGLLKPSETLSLTCAVYGGSFSNFWIGWIRQPPGKGLEWIGWINPPGSITSYADSVKGRVTISVDTSKNQFSLKLSSVTAADTAVYYCAREVGDVLDYWGQGTLVTVSS

SEQ ID NO: 170 - protein, 116 aa, synthetic construct
QVQLQQWGAGLLKPSETLSLTCAVYGGSFSSYWISWIRQPPGKGLEWIGEISPSGNTNYNPSLKSRVTISVDTSKNQFSLKLSSVTAADTAVYYCAREVGDLLDYWGQGTLVTVSS

SEQ ID NO: 171 - protein, 118 aa, synthetic construct
QVQLQQWGAGLLKPSETLSLTCAVYGGSFSSYAMNWIRQPPGKGLEWIGTISGSGGQTYYADSVKGRVTISVDTSKNQFSLKLSSVTAADTAVYYCARWRSIWAFDYWGQGTLVTVSS

SEQ ID NO: 172 - protein, 117 aa, synthetic construct
QVQLQESGPGLVKPSETLSLTCTVSGGSISSYAMSWIRQPPGKGLEWIGTITGSGGSTYYADSVKGRVTISVDTSKNQFSLKLSSVTAADTAVYYCARYKSGAFDIWGQGTLVTVSS

SEQ ID NO: 173 - protein, 117 aa, synthetic construct
QVQLQESGPGLVKPSETLSLTCTVSGGSISAYYMIWIRQPPGKGLEWIGITNPSGGVTSYAQKFQGRVTISVDTSKNQFSLKLSSVTAADTAVYYCARVGGRGFDIWGQGTLVTVSS

SEQ ID NO: 174 - protein, 116 aa, synthetic construct
QVQLQESGPGLVKPSETLSLTCTVSGGSISTYYMTWIRQPPGKGLEWIGIINPRGGSTSYAEKFQGRVTISVDTSKNQFSLKLSSVTAADTAVYYCARWNLGMDVWGQGTLVTVSS

SEQ ID NO: 175 - protein, 116 aa, synthetic construct
QVQLQESGPGLVKPSETLSLTCTVSGGSISSYGMHWIRQPPGKGLEWIGAISGSGTSIYYANSVKSRVTISVDTSKNQFSLKLSSVTAADTAVYYCARGAGWFDYWGQGTLVTVSS

SEQ ID NO: 176 - protein, 119 aa, synthetic construct
QVQLQESGPGLVKPSETLSLTCTVSGGSISTYAMSWIRQPPGKGLEWIGAISGSGGSTLYADSVKGRVTISVDTSKNQFSLKLSSVTAADTAVYYCARGGSATWAFDLWGQGTLVTVSS

SEQ ID NO: 177 - protein, 116 aa, synthetic construct
QVQLQESGPGLVKPSETLSLTCTVSGGSISTYAISWIRQPPGKGLEWIGSIYYSGYTHYNPSLESRVTISVDTSKNQFSLKLSSVTAADTAVYYCARGYSGWMDVWGQGTLVTVSS

SEQ ID NO: 178 - protein, 117 aa, synthetic construct
QVQLQESGPGLVKPSETLSLTCTVSGGSISNFWIGWIRQPPGKGLEWIGWINPPGSITSYADSVKGRVTISVDTSKNQFSLKLSSVTAADTAVYYCAREVGDVLDYWGQGTLVTVSS

SEQ ID NO: 179 - protein, 116 aa, synthetic construct
QVQLQESGPGLVKPSETLSLTCTVSGGSISSYWISWIRQPPGKGLEWIGEISPSGNTNYNPSLKSRVTISVDTSKNQFSLKLSSVTAADTAVYYCAREVGDLLDYWGQGTLVTVSS

SEQ ID NO: 180 - protein, 118 aa, synthetic construct
QVQLQESGPGLVKPSETLSLTCTVSGGSISSYAMNWIRQPPGKGLEWIGTISGSGGQTYYADSVKGRVTISVDTSKNQFSLKLSSVTAADTAVYYCARWRSIWAFDYWGQGTLVTVSS

SEQ ID NO: 181 - protein, 117 aa, synthetic construct
EVQLVQSGAEVKKPGESLKISCKGSGYSFTSYAMSWVRQMPGKGLEWMGTITGSGGSTYYADSVKGQVTISADKSISTAYLQWSSLKASDTAMYYCARYKSGAFDIWGQGTLVTVSS

SEQ ID NO: 182 - protein, 117 aa, synthetic construct
EVQLVQSGAEVKKPGESLKISCKGSGYSFTAYYMIWVRQMPGKGLEWMGITNPSGGVTSYAQKFQGQVTISADKSISTAYLQWSSLKASDTAMYYCARVGGRGFDIWGQGTLVTVSS

SEQ ID NO: 183 - protein, 116 aa, synthetic construct
EVQLVQSGAEVKKPGESLKISCKGSGYSFTTYYMTWVRQMPGKGLEWMGIINPRGGSTSYAEKFQGQVTISADKSISTAYLQWSSLKASDTAMYYCARWNLGMDVWGQGTLVTVSS

SEQ ID NO: 184 - protein, 116 aa, synthetic construct
EVQLVQSGAEVKKPGESLKISCKGSGYSFTSYGMHWVRQMPGKGLEWMGAISGSGTSIYYANSVKSQVTISADKSISTAYLQWSSLKASDTAMYYCARGAGWFDYWGQGTLVTVSS

SEQ ID NO: 185 - protein, 119 aa, synthetic construct
  REGION 1..119: note = VH
EVQLVQSGAEVKKPGESLKISCKGSGYSFTTYAMSWVRQMPGKGLEWMGAISGSGGSTLYADSVKGQVTISADKSISTAYLQWSSLKASDTAMYYCARGGSATWAFDLWGQGTLVTVSS

SEQ ID NO: 186 - protein, 116 aa, synthetic construct
EVQLVQSGAEVKKPGESLKISCKGSGYSFTTYAISWVRQMPGKGLEWMGSIYYSGYTHYNPSLESQVTISADKSISTAYLQWSSLKASDTAMYYCARGYSGWMDVWGQGTLVTVSS

SEQ ID NO: 187 - protein, 117 aa, synthetic construct
EVQLVQSGAEVKKPGESLKISCKGSGYSFTNFWIGWVRQMPGKGLEWMGWINPPGSITSYADSVKGQVTISADKSISTAYLQWSSLKASDTAMYYCAREVGDVLDYWGQGTLVTVSS

SEQ ID NO: 188 - protein, 116 aa, synthetic construct
EVQLVQSGAEVKKPGESLKISCKGSGYSFTSYWISWVRQMPGKGLEWMGEISPSGNTNYNPSLKSQVTISADKSISTAYLQWSSLKASDTAMYYCAREVGDLLDYWGQGTLVTVSS

SEQ ID NO: 189 - protein, 118 aa, synthetic construct
EVQLVQSGAEVKKPGESLKISCKGSGYSFTSYAMNWVRQMPGKGLEWMGTISGSGGQTYYADSVKGQVTISADKSISTAYLQWSSLKASDTAMYYCARWRSIWAFDYWGQGTLVTVSS

SEQ ID NO: 190 - protein, 119 aa, synthetic construct
QVQLQQSGPGLVKPSQTLSLTCAISGDSVSSYAMSWNWIRQSPSRGLEWLGTITGSGGSTYYADSVKGRITINPDTSKNQFSLQLNSVTPEDTAVYYCARYKSGAFDIWGQGTLVTVSS

SEQ ID NO: 191 - protein, 119 aa, synthetic construct
QVQLQQSGPGLVKPSQTLSLTCAISGDSVSAYYMIWNWIRQSPSRGLEWLGITNPSGGVTSYAQKFQGRITINPDTSKNQFSLQLNSVTPEDTAVYYCARVGGRGFDIWGQGTLVTVSS

SEQ ID NO: 192 - protein, 118 aa, synthetic construct
QVQLQQSGPGLVKPSQTLSLTCAISGDSVSTYYMTWNWIRQSPSRGLEWLGIINPRGGSTSYAEKFQGRITINPDTSKNQFSLQLNSVTPEDTAVYYCARWNLGMDVWGQGTLVTVSS

SEQ ID NO: 193 - protein, 118 aa, synthetic construct
QVQLQQSGPGLVKPSQTLSLTCAISGDSVSSYGMHWNWIRQSPSRGLEWLGAISGSGTSIYYANSVKSRITINPDTSKNQFSLQLNSVTPEDTAVYYCARGAGWFDYWGQGTLVTVSS

SEQ ID NO: 194 - protein, 121 aa, synthetic construct
QVQLQQSGPGLVKPSQTLSLTCAISGDSVSTYAMSWNWIRQSPSRGLEWLGAISGSGGSTLYADSVKGRITINPDTSKNQFSLQLNSVTPEDTAVYYCARGGSATWAFDLWGQGTLVTVSS

SEQ ID NO: 195 - protein, 118 aa, synthetic construct
QVQLQQSGPGLVKPSQTLSLTCAISGDSVSTYAISWNWIRQSPSRGLEWLGSIYYSGYTHYNPSLESRITINPDTSKNQFSLQLNSVTPEDTAVYYCARGYSGWMDVWGQGTLVTVSS

SEQ ID NO: 196 - protein, 120 aa, synthetic construct
QVQLQQSGPGLVKPSQTLSLTCAISGDSVSSYAMNWNWIRQSPSRGLEWLGTISGSGGQTYYADSVKGRITINPDTSKNQFSLQLNSVTPEDTAVYYCARWRSIWAFDYWGQGTLVTVSS

SEQ ID NO: 197 - protein, 118 aa, synthetic construct
QVQLQQSGPGLVKPSQTLSLTCAISGDSVSSYWISWNWIRQSPSRGLEWLGEISPSGNTNYNPSLKSRITINPDTSKNQFSLQLNSVTPEDTAVYYCAREVGDLLDYWGQGTLVTVSS

SEQ ID NO: 198 - protein, 120 aa, synthetic construct; identical to SEQ ID NO: 196

SEQ ID NO: 199 - protein, 107 aa, synthetic construct
QSVLTQPPSASGTPGQRVTISCRASQGIGNYLGWYQQLPGTAPKLLIYTASSLQSGVPDRFSGSKSGTSASLAISGLQSEDEADYYCQQGYSTPSWTFGQGTKVEIK

SEQ ID NO: 200 - protein, 106 aa, synthetic construct
QSVLTQPPSASGTPGQRVTISCHASQGISNYVAWYQQLPGTAPKLLIYDASNRATGVPDRFSGSKSGTSASLAISGLQSEDEADYYCQQSYSTLLTFGQGTKVEIK

SEQ ID NO: 201 - protein, 106 aa, synthetic construct
QSVLTQPPSASGTPGQRVTISCRVSQSISSYLNWYQQLPGTAPKLLIYDASHRATGVPDRFSGSKSGTSASLAISGLQSEDEADYYCQQYYAPSVTFGQGTKVEIK

SEQ ID NO: 202 - protein, 110 aa, synthetic construct
QSVLTQPPSASGTPGQRVTISCSGSTSNIGSNTVNWYQQLPGTAPKLLIYGKNIRPNGVPDRFSGSKSGTSASLAISGLQSEDEADYYCQSYDSSLSGWVFGGGTKLTVL

SEQ ID NO: 203 - protein, 110 aa, synthetic construct
QSVLTQPPSASGTPGQRVTISCSGSSSNIGSNYVYWYQQLPGTAPKLLIYRNNQRPSGVPDRFSGSKSGTSASLAISGLQSEDEADYYCGTWDSSLSGVVFGGGTKLTVL

SEQ ID NO: 204 - protein, 108 aa, synthetic construct
QSVLTQPPSASGTPGQRVTISCGGNNIGSKSVHWYQQLPGTAPKLLIYDNNKRPSGVPDRFSGSKSGTSASLAISGLQSEDEADYYCAAWDDSLNVPVFGGGTKLTVL

SEQ ID NO: 205 - protein, 111 aa, synthetic construct
QSVLTQPPSASGTPGQRVTISCTGTSSDIGRYNYVSWYQQLPGTAPKLLIYRNTQRPSGVPDRFSGSKSGTSASLAISGLQSEDEADYYCGTWDSSLNAYVFGGGTKLTVL

SEQ ID NO: 206 - protein, 108 aa, synthetic construct
QSVLTQPPSASGTPGQRVTISCSGSNIGNNYVSWYQQLPGTAPKLLIYQDSKRPSGVPDRFSGSKSGTSASLAISGLQSEDEADYYCLVWDRSSDHFVFGGGTKLTVL

SEQ ID NO: 207 - protein, 108 aa, synthetic construct
QSVLTQPPSASGTPGQRVTISCSDNNIGSKSVHWYQQLPGTAPKLLIYDNNKRPSGVPDRFSGSKSGTSASLAISGLQSEDEADYYCGTWDDSLSGPVFGGGTKLTVL

SEQ ID NO: 208 - protein, 107 aa, synthetic construct
QSVLTQPPSASGTPGQRVTISCRASQGIGNYLGWYQQLPGTAPKLLIYTASSLQSGVPDRFSGSKSGTSASLAISGLHSEDEADYYCQQGYSTPSWTFGQGTKVEIK

SEQ ID NO: 209 - protein, 106 aa, synthetic construct
QSVLTQPPSASGTPGQRVTISCHASQGISNYVAWYQQLPGTAPKLLIYDASNRATGVPDRFSGSKSGTSASLAISGLHSEDEADYYCQQSYSTLLTFGQGTKVEIK

SEQ ID NO: 210 - protein, 106 aa, synthetic construct
QSVLTQPPSASGTPGQRVTISCRVSQSISSYLNWYQQLPGTAPKLLIYDASHRATGVPDRFSGSKSGTSASLAISGLHSEDEADYYCQQYYAPSVTFGQGTKVEIK

SEQ ID NO: 211 - protein, 110 aa, synthetic construct
QSVLTQPPSASGTPGQRVTISCSGSTSNIGSNTVNWYQQLPGTAPKLLIYGKNIRPNGVPDRFSGSKSGTSASLAISGLHSEDEADYYCQSYDSSLSGWVFGGGTKLTVL

SEQ ID NO: 212 - protein, 110 aa, synthetic construct
QSVLTQPPSASGTPGQRVTISCSGSSSNIGSNYVYWYQQLPGTAPKLLIYRNNQRPSGVPDRFSGSKSGTSASLAISGLHSEDEADYYCGTWDSSLSGVVFGGGTKLTVL

SEQ ID NO: 213 - protein, 108 aa, synthetic construct
QSVLTQPPSASGTPGQRVTISCGGNNIGSKSVHWYQQLPGTAPKLLIYDNNKRPSGVPDRFSGSKSGTSASLAISGLHSEDEADYYCAAWDDSLNVPVFGGGTKLTVL

SEQ ID NO: 214 - protein, 111 aa, synthetic construct
QSVLTQPPSASGTPGQRVTISCTGTSSDIGRYNYVSWYQQLPGTAPKLLIYRNTQRPSGVPDRFSGSKSGTSASLAISGLHSEDEADYYCGTWDSSLNAYVFGGGTKLTVL

SEQ ID NO: 215 - protein, 108 aa, synthetic construct
QSVLTQPPSASGTPGQRVTISCSGSNIGNNYVSWYQQLPGTAPKLLIYQDSKRPSGVPDRFSGSKSGTSASLAISGLHSEDEADYYCLVWDRSSDHFVFGGGTKLTVL

SEQ ID NO: 216 - protein, 108 aa, synthetic construct; identical to SEQ ID NO: 215

SEQ ID NO: 217 - protein, 106 aa, synthetic construct
QSVLTQPPSASGTPGQRVTISCRVSQSISSYLNWYQQLPGTAPKLLIYDASHRATGVPDRFSGSKSGTSASLAISGLRSEDEADYYCQQYYAPSVTFGQGTKVEIK

SEQ ID NO: 218 - protein, 106 aa, synthetic construct
QSVLTQPPSASGTPGQRVTISCHASQGISNYVAWYQQLPGTAPKLLIYDASNRATGVPDRFSGSKSGTSASLAISGLRSEDEADYYCQQSYSTLLTFGQGTKVEIK

SEQ ID NO: 219 - protein, 106 aa, synthetic construct; identical to SEQ ID NO: 217

SEQ ID NO: 220 - protein, 110 aa, synthetic construct
QSVLTQPPSASGTPGQRVTISCSGSTSNIGSNTVNWYQQLPGTAPKLLIYGKNIRPNGVPDRFSGSKSGTSASLAISGLRSEDEADYYCQSYDSSLSGWVFGGGTKLTVL

SEQ ID NO: 221 - protein, 110 aa, synthetic construct
QSVLTQPPSASGTPGQRVTISCSGSSSNIGSNYVYWYQQLPGTAPKLLIYRNNQRPSGVPDRFSGSKSGTSASLAISGLRSEDEADYYCGTWDSSLSGVVFGGGTKLTVL

SEQ ID NO: 222 - protein, 108 aa, synthetic construct
QSVLTQPPSASGTPGQRVTISCGGNNIGSKSVHWYQQLPGTAPKLLIYDNNKRPSGVPDRFSGSKSGTSASLAISGLRSEDEADYYCAAWDDSLNVPVFGGGTKLTVL

SEQ ID NO: 223 - protein, 111 aa, synthetic construct
QSVLTQPPSASGTPGQRVTISCTGTSSDIGRYNYVSWYQQLPGTAPKLLIYRNTQRPSGVPDRFSGSKSGTSASLAISGLRSEDEADYYCGTWDSSLNAYVFGGGTKLTVL

SEQ ID NO: 224 - protein, 108 aa, synthetic construct
QSVLTQPPSASGTPGQRVTISCSGSNIGNNYVSWYQQLPGTAPKLLIYQDSKRPSGVPDRFSGSKSGTSASLAISGLRSEDEADYYCLVWDRSSDHFVFGGGTKLTVL

SEQ ID NO: 225 - protein, 108 aa, synthetic construct
QSVLTQPPSASGTPGQRVTISCSDNNIGSKSVHWYQQLPGTAPKLLIYDNNKRPSGVPDRFSGSKSGTSASLAISGLRSEDEADYYCGTWDDSLSGPVFGGGTKLTVL

SEQ ID NO: 226 - protein, 107 aa, synthetic construct
QSVLTQPPSASGTPGQRVTISCRASQGIGNYLGWYQQLPGTAPKLLIYTASSLQSGVPNRFSGSKSGTSASLAISGLRSEDEADYYCQQGYSTPSWTFGQGTKVEIK

SEQ ID NO: 227 - protein, 106 aa, synthetic construct
QSVLTQPPSASGTPGQRVTISCHASQGISNYVAWYQQLPGTAPKLLIYDASNRATGVPNRFSGSKSGTSASLAISGLRSEDEADYYCQQSYSTLLTFGQGTKVEIK

SEQ ID NO: 228 - protein, 106 aa, synthetic construct
QSVLTQPPSASGTPGQRVTISCRVSQSISSYLNWYQQLPGTAPKLLIYDASHRATGVPNRFSGSKSGTSASLAISGLRSEDEADYYCQQYYAPSVTFGQGTKVEIK

SEQ ID NO: 229 - protein, 110 aa, synthetic construct
QSVLTQPPSASGTPGQRVTISCSGSTSNIGSNTVNWYQQLPGTAPKLLIYGKNIRPNGVPNRFSGSKSGTSASLAISGLRSEDEADYYCQSYDSSLSGWVFGGGTKLTVL

SEQ ID NO: 230 - protein, 110 aa, synthetic construct
QSVLTQPPSASGTPGQRVTISCSGSSSNIGSNYVYWYQQLPGTAPKLLIYRNNQRPSGVPNRFSGSKSGTSASLAISGLRSEDEADYYCGTWDSSLSGVVFGGGTKLTVL

SEQ ID NO: 231 - protein, 108 aa, synthetic construct
QSVLTQPPSASGTPGQRVTISCGGNNIGSKSVHWYQQLPGTAPKLLIYDNNKRPSGVPNRFSGSKSGTSASLAISGLRSEDEADYYCAAWDDSLNVPVFGGGTKLTVL

SEQ ID NO: 232 - protein, 111 aa, synthetic construct
QSVLTQPPSASGTPGQRVTISCTGTSSDIGRYNYVSWYQQLPGTAPKLLIYRNTQRPSGVPNRFSGSKSGTSASLAISGLRSEDEADYYCGTWDSSLNAYVFGGGTKLTVL

SEQ ID NO: 233 - protein, 108 aa, synthetic construct
QSVLTQPPSASGTPGQRVTISCSGSNIGNNYVSWYQQLPGTAPKLLIYQDSKRPSGVPNRFSGSKSGTSASLAISGLRSEDEADYYCLVWDRSSDHFVFGGGTKLTVL

SEQ ID NO: 234 - protein, 108 aa, synthetic construct
QSVLTQPPSASGTPGQRVTISCSDNNIGSKSVHWYQQLPGTAPKLLIYDNNKRPSGVPNRFSGSKSGTSASLAISGLRSEDEADYYCGTWDDSLSGPVFGGGTKLTVL

SEQ ID NO: 235 - protein, 107 aa, synthetic construct
QSVLTQPPSVSAAPGQKVTISCRASQGIGNYLGWYQQLPGTAPKLLIYTASSLQSGIPDRFSGSKSGTSATLGITGLQTGDEADYYCQQGYSTPSWTFGQGTKVEIK

SEQ ID NO: 236 - protein, 106 aa, synthetic construct
QSVLTQPPSVSAAPGQKVTISCHASQGISNYVAWYQQLPGTAPKLLIYDASNRATGIPDRFSGSKSGTSATLGITGLQTGDEADYYCQQSYSTLLTFGQGTKVEIK

SEQ ID NO: 237 - protein, 106 aa, synthetic construct
QSVLTQPPSVSAAPGQKVTISCRVSQSISSYLNWYQQLPGTAPKLLIYDASHRATGIPDRFSGSKSGTSATLGITGLQTGDEADYYCQQYYAPSVTFGQGTKVEIK

SEQ ID NO: 238 - protein, 110 aa, synthetic construct
QSVLTQPPSVSAAPGQKVTISCSGSTSNIGSNTVNWYQQLPGTAPKLLIYGKNIRPNGIPDRFSGSKSGTSATLGITGLQTGDEADYYCQSYDSSLSGWVFGGGTKLTVL

SEQ ID NO: 239 - protein, 110 aa, synthetic construct
QSVLTQPPSVSAAPGQKVTISCSGSSSNIGSNYVYWYQQLPGTAPKLLIYRNNQRPSGIPDRFSGSKSGTSATLGITGLQTGDEADYYCGTWDSSLSGVVFGGGTKLTVL

SEQ ID NO: 240 - protein, 108 aa, synthetic construct
QSVLTQPPSVSAAPGQKVTISCGGNNIGSKSVHWYQQLPGTAPKLLIYDNNKRPSGIPDRFSGSKSGTSATLGITGLQTGDEADYYCAAWDDSLNVPVFGGGTKLTVL

SEQ ID NO: 241 - protein, 111 aa, synthetic construct
QSVLTQPPSVSAAPGQKVTISCTGTSSDIGRYNYVSWYQQLPGTAPKLLIYRNTQRPSGIPDRFSGSKSGTSATLGITGLQTGDEADYYCGTWDSSLNAYVFGGGTKLTVL

SEQ ID NO: 242 - protein, 108 aa, synthetic construct
QSVLTQPPSVSAAPGQKVTISCSGSNIGNNYVSWYQQLPGTAPKLLIYQDSKRPSGIPDRFSGSKSGTSATLGITGLQTGDEADYYCLVWDRSSDHFVFGGGTKLTVL

SEQ ID NO: 243 - protein, 108 aa, synthetic construct
QSVLTQPPSVSAAPGQKVTISCSDNNIGSKSVHWYQQLPGTAPKLLIYDNNKRPSGIPDRFSGSKSGTSATLGITGLQTGDEADYYCGTWDDSLSGPVFGGGTKLTVL

SEQ ID NO: 244 - protein, 107 aa, synthetic construct
QSALTQPASVSGSPGQSITISCRASQGIGNYLGWYQQHPGKAPKLMIYTASSLQSGVSNRFSGSKSGNTASLTISGLQAEDEADYYCQQGYSTPSWTFGQGTKVEIK

SEQ ID NO: 245 - protein, 106 aa, synthetic construct
QSALTQPASVSGSPGQSITISCHASQGISNYVAWYQQHPGKAPKLMIYDASNRATGVSNRFSGSKSGNTASLTISGLQAEDEADYYCQQSYSTLLTFGQGTKVEIK

SEQ ID NO: 246 - protein, 106 aa, synthetic construct
QSALTQPASVSGSPGQSITISCRVSQSISSYLNWYQQHPGKAPKLMIYDASHRATGVSNRFSGSKSGNTASLTISGLQAEDEADYYCQQYYAPSVTFGQGTKVEIK

SEQ ID NO: 247 - protein, 110 aa, synthetic construct
QSALTQPASVSGSPGQSITISCSGSTSNIGSNTVNWYQQHPGKAPKLMIYGKNIRPNGVSNRFSGSKSGNTASLTISGLQAEDEADYYCQSYDSSLSGWVFGGGTKLTVL

SEQ ID NO: 248 - protein, 110 aa, synthetic construct
QSALTQPASVSGSPGQSITISCSGSSSNIGSNYVYWYQQHPGKAPKLMIYRNNQRPSGVSNRFSGSKSGNTASLTISGLQAEDEADYYCGTWDSSLSGVVFGGGTKLTVL

SEQ ID NO: 249 - protein, 108 aa, synthetic construct
QSALTQPASVSGSPGQSITISCGGNNIGSKSVHWYQQHPGKAPKLMIYDNNKRPSGVSNRFSGSKSGNTASLTISGLQAEDEADYYCAAWDDSLNVPVFGGGTKLTVL

SEQ ID NO: 250 - protein, 111 aa, synthetic construct
QSALTQPASVSGSPGQSITISCTGTSSDIGRYNYVSWYQQHPGKAPKLMIYRNTQRPSGVSNRFSGSKSGNTASLTISGLQAEDEADYYCGTWDSSLNAYVFGGGTKLTVL

SEQ ID NO: 251 - protein, 108 aa, synthetic construct
QSALTQPASVSGSPGQSITISCSGSNIGNNYVSWYQQHPGKAPKLMIYQDSKRPSGVSNRFSGSKSGNTASLTISGLQAEDEADYYCLVWDRSSDHFVFGGGTKLTVL

SEQ ID NO: 252 - protein, 108 aa, synthetic construct
QSALTQPASVSGSPGQSITISCSDNNIGSKSVHWYQQHPGKAPKLMIYDNNKRPSGVSNRFSGSKSGNTASLTISGLQAEDEADYYCGTWDDSLSGPVFGGGTKLTVL

SEQ ID NO: 253 - protein, 107 aa, synthetic construct
QSALTQPRSVSGSPGQSVTISCRASQGIGNYLGWYQQHPGKAPKLMIYTASSLQSGVPDRFSGSKSGNTASLTISGLQAEDEADYYCQQGYSTPSWTFGQGTKVEIK

SEQ ID NO: 254 - protein, 106 aa, synthetic construct
QSALTQPRSVSGSPGQSVTISCHASQGISNYVAWYQQHPGKAPKLMIYDASNRATGVPDRFSGSKSGNTASLTISGLQAEDEADYYCQQSYSTLLTFGQGTKVEIK

SEQ ID NO: 255 - protein, 106 aa, synthetic construct
QSALTQPRSVSGSPGQSVTISCRVSQSISSYLNWYQQHPGKAPKLMIYDASHRATGVPDRFSGSKSGNTASLTISGLQAEDEADYYCQQYYAPSVTFGQGTKVEIK

SEQ ID NO: 256 - protein, 110 aa, synthetic construct
QSALTQPRSVSGSPGQSVTISCSGSTSNIGSNTVNWYQQHPGKAPKLMIYGKNIRPNGVPDRFSGSKSGNTASLTISGLQAEDEADYYCQSYDSSLSGWVFGGGTKLTVL

SEQ ID NO: 257 - protein, 110 aa, synthetic construct
QSALTQPRSVSGSPGQSVTISCSGSSSNIGSNYVYWYQQHPGKAPKLMIYRNNQRPSGVPDRFSGSKSGNTASLTISGLQAEDEADYYCGTWDSSLSGVVFGGGTKLTVL

SEQ ID NO: 258 - protein, 108 aa, synthetic construct
QSALTQPRSVSGSPGQSVTISCGGNNIGSKSVHWYQQHPGKAPKLMIYDNNKRPSGVPDRFSGSKSGNTASLTISGLQAEDEADYYCAAWDDSLNVPVFGGGTKLTVL

SEQ ID NO: 259 - protein, 111 aa, synthetic construct
QSALTQPRSVSGSPGQSVTISCTGTSSDIGRYNYVSWYQQHPGKAPKLMIYRNTQRPSGVPDRFSGSKSGNTASLTISGLQAEDEADYYCGTWDSSLNAYVFGGGTKLTVL

SEQ ID NO: 260 - protein, 108 aa, synthetic construct
QSALTQPRSVSGSPGQSVTISCSGSNIGNNYVSWYQQHPGKAPKLMIYQDSKRPSGVPDRFSGSKSGNTASLTISGLQAEDEADYYCLVWDRSSDHFVFGGGTKLTVL

SEQ ID NO: 261 - protein, 108 aa, synthetic construct
QSALTQPRSVSGSPGQSVTISCSDNNIGSKSVHWYQQHPGKAPKLMIYDNNKRPSGVPDRFSGSKSGNTASLTISGLQAEDEADYYCGTWDDSLSGPVFGGGTKLTVL

SEQ ID NO: 262 - protein, 107 aa, synthetic construct
SYELTQPPSVSVSPGQTASITCRASQGIGNYLGWYQQKPGQSPVLVIYTASSLQSGIPERFSGSNSGNTATLTISGTQAMDEADYYCQQGYSTPSWTFGQGTKVEIK

SEQ ID NO: 263 - protein, 106 aa, synthetic construct
SYELTQPPSVSVSPGQTASITCHASQGISNYVAWYQQKPGQSPVLVIYDASNRATGIPERFSGSNSGNTATLTISGTQAMDEADYYCQQSYSTLLTFGQGTKVEIK

SEQ ID NO: 264 - protein, 106 aa, synthetic construct
SYELTQPPSVSVSPGQTASITCRVSQSISSYLNWYQQKPGQSPVLVIYDASHRATGIPERFSGSNSGNTATLTISGTQAMDEADYYCQQYYAPSVTFGQGTKVEIK

SEQ ID NO: 265 - protein, 110 aa, synthetic construct
SYELTQPPSVSVSPGQTASITCSGSTSNIGSNTVNWYQQKPGQSPVLVIYGKNIRPNGIPERFSGSNSGNTATLTISGTQAMDEADYYCQSYDSSLSGWVFGGGTKLTVL

SEQ ID NO: 266 - protein, 110 aa, synthetic construct
SYELTQPPSVSVSPGQTASITCSGSSSNIGSNYVYWYQQKPGQSPVLVIYRNNQRPSGIPERFSGSNSGNTATLTISGTQAMDEADYYCGTWDSSLSGVVFGGGTKLTVL

SEQ ID NO: 267 - protein, 108 aa, synthetic construct
SYELTQPPSVSVSPGQTASITCGGNNIGSKSVHWYQQKPGQSPVLVIYDNNKRPSGIPERFSGSNSGNTATLTISGTQAMDEADYYCAAWDDSLNVPVFGGGTKLTVL

SEQ ID NO: 268 - protein, 111 aa, synthetic construct
SYELTQPPSVSVSPGQTASITCTGTSSDIGRYNYVSWYQQKPGQSPVLVIYRNTQRPSGIPERFSGSNSGNTATLTISGTQAMDEADYYCGTWDSSLNAYVFGGGTKLTVL

SEQ ID NO: 269 - protein, 108 aa, synthetic construct
SYELTQPPSVSVSPGQTASITCSGSNIGNNYVSWYQQKPGQSPVLVIYQDSKRPSGIPERFSGSNSGNTATLTISGTQAMDEADYYCLVWDRSSDHFVFGGGTKLTVL

SEQ ID NO: 270 - protein, 108 aa, synthetic construct
SYELTQPPSVSVSPGQTASITCSDNNIGSKSVHWYQQKPGQSPVLVIYDNNKRPSGIPERFSGSNSGNTATLTISGTQAMDEADYYCGTWDDSLSGPVFGGGTKLTVL

SEQ ID NO: 271 - protein, 108 aa, synthetic construct
DIQMTQSPSSLSASVGDRVTITCRASQGIGNYLGWYQQKPGKAPKLLIYTASSLQSGVPSRFSGSGSGTDFTFTISSLQPEDIATYYCQQGYSTPSWTFGQGTKVEIK

SEQ ID NO: 272 - protein, 107 aa, synthetic construct
DIQMTQSPSSLSASVGDRVTITCHASQGISNYVAWYQQKPGKAPKLLIYDASNRATGVPSRFSGSGSGTDFTFTISSLQPEDIATYYCQQSYSTLLTFGQGTKVEIK

SEQ ID NO: 273 - protein, 107 aa, synthetic construct
DIQMTQSPSSLSASVGDRVTITCRVSQSISSYLNWYQQKPGKAPKLLIYDASHRATGVPSRFSGSGSGTDFTFTISSLQPEDIATYYCQQYYAPSVTFGQGTKVEIK

SEQ ID NO: 274 - protein, 111 aa, synthetic construct
DIQMTQSPSSLSASVGDRVTITCSGSTSNIGSNTVNWYQQKPGKAPKLLIYGKNIRPNGVPSRFSGSGSGTDFTFTISSLQPEDIATYYCQSYDSSLSGWVFGGGTKLTVL

SEQ ID NO: 275 - protein, 111 aa, synthetic construct
DIQMTQSPSSLSASVGDRVTITCSGSSSNIGSNYVYWYQQKPGKAPKLLIYRNNQRPSGVPSRFSGSGSGTDFTFTISSLQPEDIATYYCGTWDSSLSGVVFGGGTKLTVL

SEQ ID NO: 276 - protein, 109 aa, synthetic construct
DIQMTQSPSSLSASVGDRVTITCGGNNIGSKSVHWYQQKPGKAPKLLIYDNNKRPSGVPSRFSGSGSGTDFTFTISSLQPEDIATYYCAAWDDSLNVPVFGGGTKLTVL

SEQ ID NO: 277 - protein, 112 aa, synthetic construct
DIQMTQSPSSLSASVGDRVTITCTGTSSDIGRYNYVSWYQQKPGKAPKLLIYRNTQRPSGVPSRFSGSGSGTDFTFTISSLQPEDIATYYCGTWDSSLNAYVFGGGTKLTVL

SEQ ID NO: 278 - protein, 109 aa, synthetic construct
DIQMTQSPSSLSASVGDRVTITCSGSNIGNNYVSWYQQKPGKAPKLLIYQDSKRPSGVPSRFSGSGSGTDFTFTISSLQPEDIATYYCLVWDRSSDHFVFGGGTKLTVL

SEQ ID NO: 279 - protein, 109 aa, synthetic construct
DIQMTQSPSSLSASVGDRVTITCSDNNIGSKSVHWYQQKPGKAPKLLIYDNNKRPSGVPSRFSGSGSGTDFTFTISSLQPEDIATYYCGTWDDSLSGPVFGGGTKLTVL

SEQ ID NO: 280 - protein, 108 aa, synthetic construct
DIQMTQSPSFLSASVGDRVTITCRASQGIGNYLGWYQQKPGKAPKLLIYTASSLQSGVPSRFSGSGSGTDFTLTISSLQPEDFATYYCQQGYSTPSWTFGQGTKVEIK

SEQ ID NO: 281 - protein, 107 aa, synthetic construct
DIQMTQSPSFLSASVGDRVTITCHASQGISNYVAWYQQKPGKAPKLLIYDASNRATGVPSRFSGSGSGTDFTLTISSLQPEDFATYYCQQSYSTLLTFGQGTKVEIK

SEQ ID NO: 282 - protein, 107 aa, synthetic construct
DIQMTQSPSFLSASVGDRVTITCRVSQSISSYLNWYQQKPGKAPKLLIYDASHRATGVPSRFSGSGSGTDFTLTISSLQPEDFATYYCQQYYAPSVTFGQGTKVEIK

SEQ ID NO: 283 - protein, 111 aa, synthetic construct
DIQMTQSPSFLSASVGDRVTITCSGSTSNIGSNTVNWYQQKPGKAPKLLIYGKNIRPNGVPSRFSGSGSGTDFTLTISSLQPEDFATYYCQSYDSSLSGWVFGGGTKLTVL

SEQ ID NO: 284 - protein, 111 aa, synthetic construct
DIQMTQSPSFLSASVGDRVTITCSGSSSNIGSNYVYWYQQKPGKAPKLLIYRNNQRPSGVPSRFSGSGSGTDFTLTISSLQPEDFATYYCGTWDSSLSGVVFGGGTKLTVL

SEQ ID NO: 285 - protein, 109 aa, synthetic construct
DIQMTQSPSFLSASVGDRVTITCGGNNIGSKSVHWYQQKPGKAPKLLIYDNNKRPSGVPSRFSGSGSGTDFTLTISSLQPEDFATYYCAAWDDSLNVPVFGGGTKLTVL

SEQ ID NO: 286 - protein, 112 aa, synthetic construct
DIQMTQSPSFLSASVGDRVTITCTGTSSDIGRYNYVSWYQQKPGKAPKLLIYRNTQRPSGVPSRFSGSGSGTDFTLTISSLQPEDFATYYCGTWDSSLNAYVFGGGTKLTVL

SEQ ID NO: 287 - protein, 109 aa, synthetic construct
DIQMTQSPSFLSASVGDRVTITCSGSNIGNNYVSWYQQKPGKAPKLLIYQDSKRPSGVPSRFSGSGSGTDFTLTISSLQPEDFATYYCLVWDRSSDHFVFGGGTKLTVL

SEQ ID NO: 288 - protein, 109 aa, synthetic construct
DIQMTQSPSFLSASVGDRVTITCSDNNIGSKSVHWYQQKPGKAPKLLIYDNNKRPSGVPSRFSGSGSGTDFTLTISSLQPEDFATYYCGTWDDSLSGPVFGGGTKLTVL

SEQ ID NO: 289 - protein, 108 aa, synthetic construct
DIVMTQSPLSLPVTPGEPASISCRASQGIGNYLGWYLQKPGQSPQLLIYTASSLQSGVPDRFSGSGSGTDFTLKISRVEAEDVGVYYCQQGYSTPSWTFGQGTKVEIK

SEQ ID NO: 290 - protein, 107 aa, synthetic construct
DIVMTQSPLSLPVTPGEPASISCHASQGISNYVAWYLQKPGQSPQLLIYDASNRATGVPDRFSGSGSGTDFTLKISRVEAEDVGVYYCQQSYSTLLTFGQGTKVEIK

SEQ ID NO: 291 - protein, 107 aa, synthetic construct
DIVMTQSPLSLPVTPGEPASISCRVSQSISSYLNWYLQKPGQSPQLLIYDASHRATGVPDRFSGSGSGTDFTLKISRVEAEDVGVYYCQQYYAPSVTFGQGTKVEIK

SEQ ID NO: 292 - protein, 111 aa, synthetic construct
DIVMTQSPLSLPVTPGEPASISCSGSTSNIGSNTVNWYLQKPGQSPQLLIYGKNIRPNGVPDRFSGSGSGTDFTLKISRVEAEDVGVYYCQSYDSSLSGWVFGGGTKLTVL

SEQ ID NO: 293 - protein, 111 aa, synthetic construct
DIVMTQSPLSLPVTPGEPASISCSGSSSNIGSNYVYWYLQKPGQSPQLLIYRNNQRPSGVPDRFSGSGSGTDFTLKISRVEAEDVGVYYCGTWDSSLSGVVFGGGTKLTVL

SEQ ID NO: 294 - protein, 109 aa, synthetic construct
DIVMTQSPLSLPVTPGEPASISCGGNNIGSKSVHWYLQKPGQSPQLLIYDNNKRPSGVPDRFSGSGSGTDFTLKISRVEAEDVGVYYCAAWDDSLNVPVFGGGTKLTVL

SEQ ID NO: 295 - protein, 112 aa, synthetic construct
DIVMTQSPLSLPVTPGEPASISCTGTSSDIGRYNYVSWYLQKPGQSPQLLIYRNTQRPSGVPDRFSGSGSGTDFTLKISRVEAEDVGVYYCGTWDSSLNAYVFGGGTKLTVL

SEQ ID NO: 296 - protein, 109 aa, synthetic construct
DIVMTQSPLSLPVTPGEPASISCSGSNIGNNYVSWYLQKPGQSPQLLIYQDSKRPSGVPDRFSGSGSGTDFTLKISRVEAEDVGVYYCLVWDRSSDHFVFGGGTKLTVL

SEQ ID NO: 297 - protein, 109 aa, synthetic construct
DIVMTQSPLSLPVTPGEPASISCSDNNIGSKSVHWYLQKPGQSPQLLIYDNNKRPSGVPDRFSGSGSGTDFTLKISRVEAEDVGVYYCGTWDDSLSGPVFGGGTKLTVL

SEQ ID NO: 298 - protein, 108 aa, synthetic construct
EIVMTQSPATLSVSPGERATLSCRASQGIGNYLGWYQQKPGQAPRLLIYTASSLQSGIPARFSGSGSGTEFTLTISSLQSEDFAVYYCQQGYSTPSWTFGQGTKVEIK

SEQ ID NO: 299 - protein, 107 aa, synthetic construct
EIVMTQSPATLSVSPGERATLSCHASQGISNYVAWYQQKPGQAPRLLIYDASNRATGIPARFSGSGSGTEFTLTISSLQSEDFAVYYCQQSYSTLLTFGQGTKVEIK

SEQ ID NO: 300 - protein, 107 aa, synthetic construct
EIVMTQSPATLSVSPGERATLSCRVSQSISSYLNWYQQKPGQAPRLLIYDASHRATGIPARFSGSGSGTEFTLTISSLQSEDFAVYYCQQYYAPSVTFGQGTKVEIK

SEQ ID NO: 301 - protein, 111 aa, synthetic construct
EIVMTQSPATLSVSPGERATLSCSGSTSNIGSNTVNWYQQKPGQAPRLLIYGKNIRPNGIPARFSGSGSGTEFTLTISSLQSEDFAVYYCQSYDSSLSGWVFGGGTKLTVL

SEQ ID NO: 302 - protein, 111 aa, synthetic construct
EIVMTQSPATLSVSPGERATLSCSGSSSNIGSNYVYWYQQKPGQAPRLLIYRNNQRPSGIPARFSGSGSGTEFTLTISSLQSEDFAVYYCGTWDSSLSGVVFGGGTKLTVL

SEQ ID NO: 303 - protein, 109 aa, synthetic construct
EIVMTQSPATLSVSPGERATLSCGGNNIGSKSVHWYQQKPGQAPRLLIYDNNKRPSGIPARFSGSGSGTEFTLTISSLQSEDFAVYYCAAWDDSLNVPVFGGGTKLTVL

SEQ ID NO: 304 - protein, 112 aa, synthetic construct
EIVMTQSPATLSVSPGERATLSCTGTSSDIGRYNYVSWYQQKPGQAPRLLIYRNTQRPSGIPARFSGSGSGTEFTLTISSLQSEDFAVYYCGTWDSSLNAYVFGGGTKLTVL

SEQ ID NO: 305 - protein, 109 aa, synthetic construct
EIVMTQSPATLSVSPGERATLSCSGSNIGNNYVSWYQQKPGQAPRLLIYQDSKRPSGIPARFSGSGSGTEFTLTISSLQSEDFAVYYCLVWDRSSDHFVFGGGTKLTVL

SEQ ID NO: 306 - protein, 109 aa, synthetic construct
EIVMTQSPATLSVSPGERATLSCSDNNIGSKSVHWYQQKPGQAPRLLIYDNNKRPSGIPARFSGSGSGTEFTLTISSLQSEDFAVYYCGTWDDSLSGPVFGGGTKLTVL

SEQ ID NO: 307 - protein, 108 aa, synthetic construct
EIVLTQSPGTLSLSPGERATLSCRASQGIGNYLGWYQQKPGQAPRLLIYTASSLQSGIPDRFSGSGSGTDFTLTISRLEPEDFAVYYCQQGYSTPSWTFGQGTKVEIK

SEQ ID NO: 308 - protein, 107 aa, synthetic construct
EIVLTQSPGTLSLSPGERATLSCHASQGISNYVAWYQQKPGQAPRLLIYDASNRATGIPDRFSGSGSGTDFTLTISRLEPEDFAVYYCQQSYSTLLTFGQGTKVEIK

SEQ ID NO: 309 - protein, 107 aa, synthetic construct
EIVLTQSPGTLSLSPGERATLSCRVSQSISSYLNWYQQKPGQAPRLLIYDASHRATGIPDRFSGSGSGTDFTLTISRLEPEDFAVYYCQQYYAPSVTFGQGTKVEIK

SEQ ID NO: 310 - protein, 111 aa, synthetic construct
EIVLTQSPGTLSLSPGERATLSCSGSTSNIGSNTVNWYQQKPGQAPRLLIYGKNIRPNGIPDRFSGSGSGTDFTLTISRLEPEDFAVYYCQSYDSSLSGWVFGGGTKLTVL

SEQ ID NO: 311 - protein, 111 aa, synthetic construct
EIVLTQSPGTLSLSPGERATLSCSGSSSNIGSNYVYWYQQKPGQAPRLLIYRNNQRPSGIPDRFSGSGSGTDFTLTISRLEPEDFAVYYCGTWDSSLSGVVFGGGTKLTVL

SEQ ID NO: 312 - protein, 109 aa, synthetic construct
EIVLTQSPGTLSLSPGERATLSCGGNNIGSKSVHWYQQKPGQAPRLLIYDNNKRPSGIPDRFSGSGSGTDFTLTISRLEPEDFAVYYCAAWDDSLNVPVFGGGTKLTVL

SEQ ID NO: 313 - protein, 112 aa, synthetic construct
EIVLTQSPGTLSLSPGERATLSCTGTSSDIGRYNYVSWYQQKPGQAPRLLIYRNTQRPSGIPDRFSGSGSGTDFTLTISRLEPEDFAVYYCGTWDSSLNAYVFGGGTKLTVL

SEQ ID NO: 314 - protein, 109 aa, synthetic construct
EIVLTQSPGTLSLSPGERATLSCSGSNIGNNYVSWYQQKPGQAPRLLIYQDSKRPSGIPDRFSGSGSGTDFTLTISRLEPEDFAVYYCLVWDRSSDHFVFGGGTKLTVL

SEQ ID NO: 315 - protein, 109 aa, synthetic construct
EIVLTQSPGTLSLSPGERATLSCSDNNIGSKSVHWYQQKPGQAPRLLIYDNNKRPSGIPDRFSGSGSGTDFTLTISRLEPEDFAVYYCGTWDDSLSGPVFGGGTKLTVL

SEQ ID NO: 316 - protein, 108 aa, synthetic construct
EIVLTQSPGTLSLSPGERATLSCRASQGIGNYLGWYQQKPGQAPRLLIYTASSLQSGIPDRFSGSGSGTDFTLTISHLEPEDFAVYYCQQGYSTPSWTFGQGTKVEIK

SEQ ID NO: 317 - protein, 107 aa, synthetic construct
EIVLTQSPGTLSLSPGERATLSCHASQGISNYVAWYQQKPGQAPRLLIYDASNRATGIPDRFSGSGSGTDFTLTISHLEPEDFAVYYCQQSYSTLLTFGQGTKVEIK

SEQ ID NO: 318 - protein, 107 aa, synthetic construct
EIVLTQSPGTLSLSPGERATLSCRVSQSISSYLNWYQQKPGQAPRLLIYDASHRATGIPDRFSGSGSGTDFTLTISHLEPEDFAVYYCQQYYAPSVTFGQGTKVEIK

SEQ ID NO: 319 - protein, 111 aa, synthetic construct
EIVLTQSPGTLSLSPGERATLSCSGSTSNIGSNTVNWYQQKPGQAPRLLIYGKNIRPNGIPDRFSGSGSGTDFTLTISHLEPEDFAVYYCQSYDSSLSGWVFGGGTKLTVL

SEQ ID NO: 320 - protein, 111 aa, synthetic construct
EIVLTQSPGTLSLSPGERATLSCSGSSSNIGSNYVYWYQQKPGQAPRLLIYRNNQRPSGIPDRFSGSGSGTDFTLTISHLEPEDFAVYYCGTWDSSLSGVVFGGGTKLTVL

SEQ ID NO: 321 - protein, 109 aa, synthetic construct
EIVLTQSPGTLSLSPGERATLSCGGNNIGSKSVHWYQQKPGQAPRLLIYDNNKRPSGIPDRFSGSGSGTDFTLTISHLEPEDFAVYYCAAWDDSLNVPVFGGGTKLTVL

SEQ ID NO: 322 - protein, 112 aa, synthetic construct
EIVLTQSPGTLSLSPGERATLSCTGTSSDIGRYNYVSWYQQKPGQAPRLLIYRNTQRPSGIPDRFSGSGSGTDFTLTISHLEPEDFAVYYCGTWDSSLNAYVFGGGTKLTVL

SEQ ID NO: 323 - protein, 109 aa, synthetic construct
EIVLTQSPGTLSLSPGERATLSCSGSNIGNNYVSWYQQKPGQAPRLLIYQDSKRPSGIPDRFSGSGSGTDFTLTISHLEPEDFAVYYCLVWDRSSDHFVFGGGTKLTVL

SEQ ID NO: 324 - protein, 109 aa, synthetic construct
EIVLTQSPGTLSLSPGERATLSCSDNNIGSKSVHWYQQKPGQAPRLLIYDNNKRPSGIPDRFSGSGSGTDFTLTISHLEPEDFAVYYCGTWDDSLSGPVFGGGTKLTVL

SEQ ID NO: 325 - protein, 108 aa, synthetic construct
DIVMTQSPDSLAVSLGERATINCRASQGIGNYLGWYQQKPGQPPKLLIYTASSLQSGVPDRFSGSGSGTDFTLTISSLQAEDVAVYYCQQGYSTPSWTFGQGTKVEIK

SEQ ID NO: 326 - protein, 107 aa, synthetic construct
DIVMTQSPDSLAVSLGERATINCHASQGISNYVAWYQQKPGQPPKLLIYDASNRATGVPDRFSGSGSGTDFTLTISSLQAEDVAVYYCQQSYSTLLTFGQGTKVEIK

SEQ ID NO: 327 - protein, 107 aa, synthetic construct
DIVMTQSPDSLAVSLGERATINCRVSQSISSYLNWYQQKPGQPPKLLIYDASHRATGVPDRFSGSGSGTDFTLTISSLQAEDVAVYYCQQYYAPSVTFGQGTKVEIK

SEQ ID NO: 328 - protein, 111 aa, synthetic construct
DIVMTQSPDSLAVSLGERATINCSGSTSNIGSNTVNWYQQKPGQPPKLLIYGKNIRPNGVPDRFSGSGSGTDFTLTISSLQAEDVAVYYCQSYDSSLSGWVFGGGTKLTVL

SEQ ID NO: 329 - protein, 111 aa, synthetic construct
DIVMTQSPDSLAVSLGERATINCSGSSSNIGSNYVYWYQQKPGQPPKLLIYRNNQRPSGVPDRFSGSGSGTDFTLTISSLQAEDVAVYYCGTWDSSLSGVVFGGGTKLTVL

SEQ ID NO: 330 - protein, 109 aa, synthetic construct
DIVMTQSPDSLAVSLGERATINCGGNNIGSKSVHWYQQKPGQPPKLLIYDNNKRPSGVPDRFSGSGSGTDFTLTISSLQAEDVAVYYCAAWDDSLNVPVFGGGTKLTVL

SEQ ID NO: 331 - protein, 112 aa, synthetic construct
DIVMTQSPDSLAVSLGERATINCTGTSSDIGRYNYVSWYQQKPGQPPKLLIYRNTQRPSGVPDRFSGSGSGTDFTLTISSLQAEDVAVYYCGTWDSSLNAYVFGGGTKLTVL

SEQ ID NO: 332 - protein, 109 aa, synthetic construct
DIVMTQSPDSLAVSLGERATINCSGSNIGNNYVSWYQQKPGQPPKLLIYQDSKRPSGVPDRFSGSGSGTDFTLTISSLQAEDVAVYYCLVWDRSSDHFVFGGGTKLTVL

SEQ ID NO: 333 - protein, 109 aa, synthetic construct
DIVMTQSPDSLAVSLGERATINCSDNNIGSKSVHWYQQKPGQPPKLLIYDNNKRPSGVPDRFSGSGSGTDFTLTISSLQAEDVAVYYCGTWDDSLSGPVFGGGTKLTVL

SEQ ID NO: 334 - protein, 11 aa, synthetic construct
WGQGTLVTVSS

SEQ ID NO: 335 - protein, 10 aa, synthetic construct
FGQGTKVEIK

SEQ ID NO: 336 - protein, 10 aa, synthetic construct
FGGGTKLTVL

SEQ ID NO: 337 - protein, 137 aa, synthetic construct
TIPPHVQKSVNNDMIVTDNNGAVKFPQLCKFCDVRFSTCDNQKSCMSNCSITSICEKPQEVCVAVWRKNDENITLETVCHDPKLPYHDFILEDAASPKCIMKEKKKPGETFFMCSCSSDECNDNIIFSEEYNTSNPD

SEQ ID NO: 338 - protein, 15 aa, synthetic construct
GGGGSGGGGSGGGGS

SEQ ID NO: 339 - protein, 599 aa, synthetic construct
EVQLLESGGGLVQPGGSLRLSCAASGFTFSSYAMSWVRQAPGKGLEWVSTITGSGGSTYYADSVKGRFTISRDNSKNTLYLQMNSLRAEDTAVYYCARYKSGAFDIWGQGTLVTVSSASTKGPSVFPLAPSSKSTSGGTAALGCLVKDYFPEPVTVSWNSGALTSGVHTFPAVLQSSGLYSLSSVVTVPSSSLGTQTYICNVNHKPSNTKVDKKVEPKSCDKTHTCPPCPAPELLGGPSVFLFPPKPKDTLMISRTPEVTCVVVDVSHEDPEVKFNWYVDGVEVHNAKTKPREEQYASTYRVVSVLTVLHQDWLNGKEYKCKVSNKALPAPIEKTISKAKGQPREPQVYTLPPSREEMTKNQVSLTCLVKGFYPSDIAVEWESNGQPENNYKTTPPVLDSDGSFFLYSKLTVDKSRWQQGNVFSCSVMHEALHNHYTQKSLSLSPGKGGGGSGGGGSGGGGSTIPPHVQKSVNNDMIVTDNNGAVKFPQLCKFCDVRFSTCDNQKSCMSNCSITSICEKPQEVCVAVWRKNDENITLETVCHDPKLPYHDFILEDAASPKCIMKEKKKPGETFFMCSCSSDECNDNIIFSEEYNTSNPD

SEQ ID NO: 340 - protein, 599 aa, synthetic construct
EVQLLESGGGLVQPGGSLRLSCAASGFTFSAYYMIWVRQAPGKGLEWVSITNPSGGVTSYAQKFQGRFTISRDNSKNTLYLQMNSLRAEDTAVYYCARVGGRGFDIWGQGTLVTVSSASTKGPSVFPLAPSSKSTSGGTAALGCLVKDYFPEPVTVSWNSGALTSGVHTFPAVLQSSGLYSLSSVVTVPSSSLGTQTYICNVNHKPSNTKVDKKVEPKSCDKTHTCPPCPAPELLGGPSVFLFPPKPKDTLMISRTPEVTCVVVDVSHEDPEVKFNWYVDGVEVHNAKTKPREEQYASTYRVVSVLTVLHQDWLNGKEYKCKVSNKALPAPIEKTISKAKGQPREPQVYTLPPSREEMTKNQVSLTCLVKGFYPSDIAVEWESNGQPENNYKTTPPVLDSDGSFFLYSKLTVDKSRWQQGNVFSCSVMHEALHNHYTQKSLSLSPGKGGGGSGGGGSGGGGSTIPPHVQKSVNNDMIVTDNNGAVKFPQLCKFCDVRFSTCDNQKSCMSNCSITSICEKPQEVCVAVWRKNDENITLETVCHDPKLPYHDFILEDAASPKCIMKEKKKPGETFFMCSCSSDECNDNIIFSEEYNTSNPD

SEQ ID NO: 341 - protein, 598 aa, synthetic construct
EVQLLESGGGLVQPGGSLRLSCAASGFTFSTYYMTWVRQAPGKGLEWVSIINPRGGSTSYAEKFQGRFTISRDNSKNTLYLQMNSLRAEDTAVYYCARWNLGMDVWGQGTLVTVSSASTKGPSVFPLAPSSKSTSGGTAALGCLVKDYFPEPVTVSWNSGALTSGVHTFPAVLQSSGLYSLSSVVTVPSSSLGTQTYICNVNHKPSNTKVDKKVEPKSCDKTHTCPPCPAPELLGGPSVFLFPPKPKDTLMISRTPEVTCVVVDVSHEDPEVKFNWYVDGVEVHNAKTKPREEQYASTYRVVSVLTVLHQDWLNGKEYKCKVSNKALPAPIEKTISKAKGQPREPQVYTLPPSREEMTKNQVSLTCLVKGFYPSDIAVEWESNGQPENNYKTTPPVLDSDGSFFLYSKLTVDKSRWQQGNVFSCSVMHEALHNHYTQKSLSLSPGKGGGGSGGGGSGGGGSTIPPHVQKSVNNDMIVTDNNGAVKFPQLCKFCDVRFSTCDNQKSCMSNCSITSICEKPQEVCVAVWRKNDENITLETVCHDPKLPYHDFILEDAASPKCIMKEKKKPGETFFMCSCSSDECNDNIIFSEEYNTSNPD

SEQ ID NO: 342 - protein, 598 aa, synthetic construct
EVQLLESGGGLVQPGGSLRLSCAASGFTFSSYGMHWVRQAPGKGLEWVSAISGSGTSIYYANSVKSRFTISRDNSKNTLYLQMNSLRAEDTAVYYCARGAGWFDYWGQGTLVTVSSASTKGPSVFPLAPSSKSTSGGTAALGCLVKDYFPEPVTVSWNSGALTSGVHTFPAVLQSSGLYSLSSVVTVPSSSLGTQTYICNVNHKPSNTKVDKKVEPKSCDKTHTCPPCPAPELLGGPSVFLFPPKPKDTLMISRTPEVTCVVVDVSHEDPEVKFNWYVDGVEVHNAKTKPREEQYASTYRVVSVLTVLHQDWLNGKEYKCKVSNKALPAPIEKTISKAKGQPREPQVYTLPPSREEMTKNQVSLTCLVKGFYPSDIAVEWESNGQPENNYKTTPPVLDSDGSFFLYSKLTVDKSRWQQGNVFSCSVMHEALHNHYTQKSLSLSPGKGGGGSGGGGSGGGGSTIPPHVQKSVNNDMIVTDNNGAVKFPQLCKFCDVRFSTCDNQKSCMSNCSITSICEKPQEVCVAVWRKNDENITLETVCHDPKLPYHDFILEDAASPKCIMKEKKKPGETFFMCSCSSDECNDNIIFSEEYNTSNPD

SEQ ID NO: 343 - protein, 601 aa, synthetic construct
EVQLLESGGGLVQPGGSLRLSCAASGFTFSTYAMSWVRQAPGKGLEWVSAISGSGGSTLYADSVKGRFTISRDNSKNTLYLQMNSLRAEDTAVYYCARGGSATWAFDLWGQGTLVTVSSASTKGPSVFPLAPSSKSTSGGTAALGCLVKDYFPEPVTVSWNSGALTSGVHTFPAVLQSSGLYSLSSVVTVPSSSLGTQTYICNVNHKPSNTKVDKKVEPKSCDKTHTCPPCPAPELLGGPSVFLFPPKPKDTLMISRTPEVTCVVVDVSHEDPEVKFNWYVDGVEVHNAKTKPREEQYASTYRVVSVLTVLHQDWLNGKEYKCKVSNKALPAPIEKTISKAKGQPREPQVYTLPPSREEMTKNQVSLTCLVKGFYPSDIAVEWESNGQPENNYKTTPPVLDSDGSFFLYSKLTVDKSRWQQGNVFSCSVMHEALHNHYTQKSLSLSPGKGGGGSGGGGSGGGGSTIPPHVQKSVNNDMIVTDNNGAVKFPQLCKFCDVRFSTCDNQKSCMSNCSITSICEKPQEVCVAVWRKNDENITLETVCHDPKLPYHDFILEDAASPKCIMKEKKKPGETFFMCSCSSDECNDNIIFSEEYNTSNPD

SEQ ID NO: 344 - protein, 598 aa, synthetic construct
EVQLLESGGGLVQPGGSLRLSCAASGFTFSTYAISWVRQAPGKGLEWVSSIYYSGYTHYNPSLESRFTISRDNSKNTLYLQMNSLRAEDTAVYYCARGYSGWMDVWGQGTLVTVSSASTKGPSVFPLAPSSKSTSGGTAALGCLVKDYFPEPVTVSWNSGALTSGVHTFPAVLQSSGLYSLSSVVTVPSSSLGTQTYICNVNHKPSNTKVDKKVEPKSCDKTHTCPPCPAPELLGGPSVFLFPPKPKDTLMISRTPEVTCVVVDVSHEDPEVKFNWYVDGVEVHNAKTKPREEQYASTYRVVSVLTVLHQDWLNGKEYKCKVSNKALPAPIEKTISKAKGQPREPQVYTLPPSREEMTKNQVSLTCLVKGFYPSDIAVEWESNGQPENNYKTTPPVLDSDGSFFLYSKLTVDKSRWQQGNVFSCSVMHEALHNHYTQKSLSLSPGKGGGGSGGGGSGGGGSTIPPHVQKSVNNDMIVTDNNGAVKFPQLCKFCDVRFSTCDNQKSCMSNCSITSICEKPQEVCVAVWRKNDENITLETVCHDPKLPYHDFILEDAASPKCIMKEKKKPGETFFMCSCSSDECNDNIIFSEEYNTSNPD

SEQ ID NO: 345 - protein, 599 aa, synthetic construct
EVQLLESGGGLVQPGGSLRLSCAASGFTFSNFWIGWVRQAPGKGLEWVSWINPPGSITSYADSVKGRFTISRDNSKDTLYLQMNSLRAEDTAVYYCAREVGDVLDYWGQGTLVTVSSASTKGPSVFPLAPSSKSTSGGTAALGCLVKDYFPEPVTVSWNSGALTSGVHTFPAVLQSSGLYSLSSVVTVPSSSLGTQTYICNVNHKPSNTKVDKKVEPKSCDKTHTCPPCPAPELLGGPSVFLFPPKPKDTLMISRTPEVTCVVVDVSHEDPEVKFNWYVDGVEVHNAKTKPREEQYASTYRVVSVLTVLHQDWLNGKEYKCKVSNKALPAPIEKTISKAKGQPREPQVYTLPPSREEMTKNQVSLTCLVKGFYPSDIAVEWESNGQPENNYKTTPPVLDSDGSFFLYSKLTVDKSRWQQGNVFSCSVMHEALHNHYTQKSLSLSPGKGGGGSGGGGSGGGGSTIPPHVQKSVNNDMIVTDNNGAVKFPQLCKFCDVRFSTCDNQKSCMSNCSITSICEKPQEVCVAVWRKNDENITLETVCHDPKLPYHDFILEDAASPKCIMKEKKKPGETFFMCSCSSDECNDNIIFSEEYNTSNPD

SEQ ID NO: 346 - protein, 598 aa, synthetic construct
EVQLLESGGGLVQPGSSLRLSCAASGFTFSSYWISWVRQAPGKGLEWVSEISPSGNTNYNPSLKSRFTISRDNSKNTLYLQMNSLRAEDTAVYYCAREVGDLLDYWGQGTLVTVSSASTKGPSVFPLAPSSKSTSGGTAALGCLVKDYFPEPVTVSWNSGALTSGVHTFPAVLQSSGLYSLSSVVTVPSSSLGTQTYICNVNHKPSNTKVDKKVEPKSCDKTHTCPPCPAPELLGGPSVFLFPPKPKDTLMISRTPEVTCVVVDVSHEDPEVKFNWYVDGVEVHNAKTKPREEQYASTYRVVSVLTVLHQDWLNGKEYKCKVSNKALPAPIEKTISKAKGQPREPQVYTLPPSREEMTKNQVSLTCLVKGFYPSDIAVEWESNGQPENNYKTTPPVLDSDGSFFLYSKLTVDKSRWQQGNVFSCSVMHEALHNHYTQKSLSLSPGKGGGGSGGGGSGGGGSTIPPHVQKSVNNDMIVTDNNGAVKFPQLCKFCDVRFSTCDNQKSCMSNCSITSICEKPQEVCVAVWRKNDENITLETVCHDPKLPYHDFILEDAASPKCIMKEKKKPGETFFMCSCSSDECNDNIIFSEEYNTSNPD

SEQ ID NO: 347 - protein, 600 aa, synthetic construct
EVQLLESGGGLVQPGGSLRLSCAASGFTFSSYAMNWVRQAPGKGLEWVSTISGSGGQTYYADSVKGRFTISRDNSKNTLYLQMNSLRAEDTAVYYCARWRSIWAFDYWGQGTLVTVSSASTKGPSVFPLAPSSKSTSGGTAALGCLVKDYFPEPVTVSWNSGALTSGVHTFPAVLQSSGLYSLSSVVTVPSSSLGTQTYICNVNHKPSNTKVDKKVEPKSCDKTHTCPPCPAPELLGGPSVFLFPPKPKDTLMISRTPEVTCVVVDVSHEDPEVKFNWYVDGVEVHNAKTKPREEQYASTYRVVSVLTVLHQDWLNGKEYKCKVSNKALPAPIEKTISKAKGQPREPQVYTLPPSREEMTKNQVSLTCLVKGFYPSDIAVEWESNGQPENNYKTTPPVLDSDGSFFLYSKLTVDKSRWQQGNVFSCSVMHEALHNHYTQKSLSLSPGKGGGGSGGGGSGGGGSTIPPHVQKSVNNDMIVTDNNGAVKFPQLCKFCDVRFSTCDNQKSCMSNCSITSICEKPQEVCVAVWRKNDENITLETVCHDPKLPYHDFILEDAASPKCIMKEKKKPGETFFMCSCSSDECNDNIIFSEEYNTSNPD

SEQ ID NO: 348 - protein, 330 aa, synthetic construct
ASTKGPSVFPLAPSSKSTSGGTAALGCLVKDYFPEPVTVSWNSGALTSGVHTFPAVLQSSGLYSLSSVVTVPSSSLGTQTYICNVNHKPSNTKVDKKVEPKSCDKTHTCPPCPAPELLGGPSVFLFPPKPKDTLMISRTPEVTCVVVDVSHEDPEVKFNWYVDGVEVHNAKTKPREEQYASTYRVVSVLTVLHQDWLNGKEYKCKVSNKALPAPIEKTISKAKGQPREPQVYTLPPSREEMTKNQVSLTCLVKGFYPSDIAVEWESNGQPENNYKTTPPVLDSDGSFFLYSKLTVDKSRWQQGNVFSCSVMHEALHNHYTQKSLSLSPGK